European Patent Application EP 4 755 387 A2, published June 10, 2026. Title: NUCLEOTIDE DERIVATIVES AND METHODS OF USE THEREOF. Applicant: THE TRUSTEES OF COLUMBIA UNIVERSITY IN THE CITY OF NEW YORK. The sequence listing filed with the application follows.

SEQUENCE LISTING (27 sequences)

SEQ ID NO: 1 - DNA, 109 bp, Homo sapiens
  source 1..109: mol_type = unassigned DNA
gaaggagacacgcggccagagagggtcctgtccgtgtttgtgcgtggagttcgacaaggcagggtcatctaatggtgatgagtcctatccttttctcttcgttctccgt

SEQ ID NO: 2 - DNA, 20 bp, Homo sapiens
  source 1..20: mol_type = unassigned DNA
tagatgaccctgccttgtcg

SEQ ID NO: 3 - DNA, 109 bp, Homo sapiens; identical to SEQ ID NO: 1
  source 1..109: mol_type = unassigned DNA

SEQ ID NO: 4 - DNA, 17 bp, Homo sapiens
  source 1..17: mol_type = unassigned DNA
gataggactcatcacca

SEQ ID NO: 5 - DNA, 109 bp, Homo sapiens; identical to SEQ ID NO: 1
  source 1..109: mol_type = unassigned DNA

SEQ ID NO: 6 - DNA, 109 bp, Homo sapiens
  source 1..109: mol_type = unassigned DNA
gaaggagacacgcggccagagagggtcctgtccgtgtttgtccgtggagttcgacaaggcagggtcatctaatggtgatgagtcctatccttttctcttcgttctccgt

SEQ ID NO: 7 - DNA, 20 bp, Homo sapiens
  source 1..20: mol_type = unassigned DNA
tagatgaccctgccttgtcg

SEQ ID NO: 8 - DNA, 109 bp, Homo sapiens; identical to SEQ ID NO: 6
  source 1..109: mol_type = unassigned DNA

SEQ ID NO: 9 - DNA, 20 bp, Homo sapiens
  source 1..20: mol_type = unassigned DNA
tagatgaccctgccttgtcg

SEQ ID NO: 10 - DNA, 109 bp, Homo sapiens; identical to SEQ ID NO: 6
  source 1..109: mol_type = unassigned DNA

SEQ ID NO: 11 - DNA, 20 bp, Homo sapiens
  source 1..20: mol_type = unassigned DNA
tagatgaccctgccttgtcg

SEQ ID NO: 12 - DNA, 109 bp, Homo sapiens; identical to SEQ ID NO: 6
  source 1..109: mol_type = unassigned DNA

SEQ ID NO: 13 - DNA, 17 bp, Homo sapiens
  source 1..17: mol_type = unassigned DNA
gataggactcatcacca

SEQ ID NO: 14 - DNA, 100 bp, Homo sapiens
  source 1..100: mol_type = unassigned DNA
tacccggaggccaagtacggcgggtacgtccttgacaatgtgtacatcaacatcacctaccaccatgtcagtctcggttggatcctctattgtgtccggg

SEQ ID NO: 15 - DNA, 20 bp, Homo sapiens
  source 1..20: mol_type = unassigned DNA
gttgatgtacacattgtcaa

SEQ ID NO: 16 - DNA, 109 bp, Homo sapiens; identical to SEQ ID NO: 6
  source 1..109: mol_type = unassigned DNA

SEQ ID NO: 17 - DNA, 20 bp, Homo sapiens
  source 1..20: mol_type = unassigned DNA
tagatgaccctgccttgtcg

SEQ ID NO: 18 - DNA, 20 bp, Homo sapiens
  source 1..20: mol_type = unassigned DNA
tagatgaccctgccttgtcg

SEQ ID NO: 19 - DNA, 109 bp, Homo sapiens; identical to SEQ ID NO: 1
  source 1..109: mol_type = unassigned DNA

SEQ ID NO: 20 - DNA, 20 bp, Homo sapiens
  source 1..20: mol_type = unassigned DNA
tagatgaccctgccttgtcg

SEQ ID NO: 21 - DNA, 109 bp, Homo sapiens; identical to SEQ ID NO: 1
  source 1..109: mol_type = unassigned DNA

SEQ ID NO: 22 - DNA, 17 bp, Homo sapiens
  source 1..17: mol_type = unassigned DNA
gataggactcatcacca

SEQ ID NO: 23 - DNA, 109 bp, Homo sapiens; identical to SEQ ID NO: 1
  source 1..109: mol_type = unassigned DNA

SEQ ID NO: 24 - DNA, 51 bp, Homo sapiens
  source 1..51: mol_type = unassigned DNA
tacatcaactacccggaggccaagtacggcgggtacgtccttgacaatgtg

SEQ ID NO: 25 - DNA, 13 bp, Homo sapiens
  source 1..13: mol_type = unassigned DNA
cacattgtcaagg

SEQ ID NO: 26 - DNA, 80 bp, Homo sapiens
  source 1..80: mol_type = unassigned DNA
gaggaagtatcctgtcgtttagcatacccaaacttgatgctctactgacctcagctgcacgtaagtgcagctgaggtcag

SEQ ID NO: 27 - DNA, 80 bp, Homo sapiens
  source 1..80: mol_type = unassigned DNA
tcacagaggaagtatcctgtcgtttagcatacccaaacttgatgctgacctcagctgcacgtaagtgcagctgaggtcag